European Patent Application EP 4 198 134 A1, published June 21, 2023. Title: GAMMA-SARCOGLYCAN GENE TRANSFER INCREASE USING MODIFIED ITR SEQUENCES. Applicant: GENETHON INSTITUT NATIONAL DE LA SANTE ET DE LA RECHERCHE MEDICALE UNIVERSITE D'EVRY VAL D’ESSONNE. The sequence listing filed with the application follows.

SEQUENCE LISTING (11 sequences)

SEQ ID NO: 1 - DNA, 108 bp, Artificial Sequence
  ITRg 5' (22 bp - deleted)
ctgcgcgctcgctcgctcactgaggccgcccgggcaaagcccgggcggcctcagtgagcgagcgagcgcgcagagagggagtggccaactccatcactaggggttcct

SEQ ID NO: 2 - DNA, 130 bp, Artificial Sequence
  ITRg 3'
aggaacccctagtgatggagttggccactccctctctgcgcgctcgctcgctcactgaggccgggcgaccaaaggtcgcccgacgcccgggctttgcccgggcggcctcagtgagcgagcgagcgcgcag

SEQ ID NO: 3 - DNA, 876 bp, Artificial Sequence
  SGCG WT
atggtgcgtgagcagtacactacagccacagaaggcatctgcatagagaggccagagaatcagtatgtctacaaaattggcatttatggctggagaaagcgctgtctctacttgtttgttcttcttttactcatcatcctcgttgtgaatttagctcttacaatttggattcttaaagtgatgtggttttctccagcaggaatgggccacttgtgtgtaacaaaagatggactgcgcttggaaggggaatcagaatttttattcccattgtatgccaaagaaatacactccagagtggactcatctctgctgctacaatcaacccagaatgtgactgtaaatgcgcgcaactcagaaggggaggtcacaggcaggttaaaagtcggtcccaaaatggtagaagtccagaatcaacagtttcagatcaactccaacgacggcaagccactatttactgtagatgagaaggaagttgtggttggtacagataaacttcgagtaactgggcctgaaggggctctttttgaacattcagtggagacaccccttgtcagagccgacccgtttcaagaccttagattagaatcccccactcggagtctaagcatggatgccccaaggggtgtgcatattcaagctcacgctgggaaaattgaggcgctttctcaaatggatattctttttcatagtagtgatggaatgctcgtgcttgatgctgaaactgtgtgcttacccaagctggtgcaggggacgtggggtccctctggcagctcacagagcctctacgaaatctgtgtgtgtccagatgggaagctgtacctgtctgtggccggtgtgagcaccacgtgccaggagcacagccacatctgcctctaa

SEQ ID NO: 4 - DNA, 1061 bp, Artificial Sequence
  Human Desmin Promoter
taccccctgccccccacagctcctctcctgtgccttgtttcccagccatgcgttctcctctataaatacccgctctggtatttggggttggcagctgttgctgccagggagatggttgggttgacatgcggctcctgacaaaacacaaacccctggtgtgtgtgggcgtgggtggtgtgagtagggggatgaatcagggagggggcgggggacccagggggcaggagccacacaaagtctgtgcgggggtgggagcgcacatagcaattggaaactgaaagcttatcagaccctttctggaaatcagcccactgtttataaacttgaggccccaccctcgacagtaccggggaggaagagggcctgcactagtccagagggaaactgaggctcagggctagctcgcccatagacatacatggcaggcaggctttggccaggatccctccgcctgccaggcgtctccctgccctcccttcctgcctagagacccccaccctcaagcctggctggtctttgcctgagacccaaacctcttcgacttcaagagaatatttaggaacaaggtggtttagggcctttcctgggaacaggccttgaccctttaagaaatgacccaaagtctctccttgaccaaaaaggggaccctcaaactaaagggaagcctctcttctgctgtctcccctgaccccactcccccccaccccaggacgaggagataaccagggctgaaagaggcccgcctgggggctgcagacatgcttgctgcctgccctggcgaaggattggcaggcttgcccgtcacaggacccccgctggctgactcaggggcgcaggcctcttgcgggggagctggcctccccgcccccacggccacgggccgccctttcctggcaggacagcgggatcttgcagctgtcaggggaggggaggcgggggctgatgtcaggagggatacaaatagtgccgacggctgggggccctgtctcccctcgccgcatccactctccggccggccgcctgcccgccgcctcctccgtgcgcccgccagcctcgcccgc

SEQ ID NO: 5 - DNA, 762 bp, Artificial Sequence
  pA-HBB2
accccaccagtgcaggctgcctatcagaaagtggtggctggtgtggctaatgccctggcccacaagtatcactaagctcgctttcttgctgtccaatttctattaaaggttcctttgttccctaagtccaactactaaactgggggatattatgaagggccttgagcatctggattctgcctaataaaaaacatttattttcattgcaatgatgtatttaaattatttctgaatattttactaaaaagggaatgtgggaggtcagtgcatttaaaacataaagaaatgaagagctagttcaaaccttgggaaaatacactatatcttaaactccatgaaagaaggtgaggctgcaaacagctaatgcacattggcaacagccctgatgcctatgccttattcatccctcagaaaaggattcaagtagaggcttgatttggaggttaaagttttgctatgctgtattttacattacttattgttttagctgtcctcatgaatgtcttttcactacccatttgcttatcctgcatctctcagccttgactccactcagttctcttgcttagagataccacctttcccctgaagtgttccttccatgttttacggcgagatggtttctcctcgcctggccactcagccttagttgtctctgttgtcttatagaggtctacttgaagaaggaaaaacagggggcatggtttgactgtcctgtgagcccttcttccctgcctcccccactcacagtgacccggaatc

SEQ ID NO: 6 - DNA, 18 bp, Artificial Sequence
  polyA HBB2 sequence FWD
ccaggcgaggagaaacca

SEQ ID NO: 7 - DNA, 25 bp, Artificial Sequence
  polyA HBB2 sequence REV
cttgactccactcagttctcttgct

SEQ ID NO: 8 - DNA, 29 bp, Artificial Sequence
  polyA HBB2 sequence Probe
ctcgccgtaaaacatggaaggaacacttc

SEQ ID NO: 9 - DNA, 20 bp, Artificial Sequence
  ribosomal phosphoprotein FWD
ctccaagcagatgcagcaga

SEQ ID NO: 10 - DNA, 20 bp, Artificial Sequence
  ribosomal phosphoprotein REV
atagccttgcgcatcatggt

SEQ ID NO: 11 - DNA, 22 bp, Artificial Sequence
  ribosomal phosphoprotein Probe
ccgtggtgctgatgggcaagaa